European Patent Specification EP 3 016 504 B1, published May 24, 2023. Title: PEPPER WITH INCREASED BRIX LEVEL. Applicant: Rijk Zwaan Zaadteelt en Zaadhandel B.V. The sequence listing filed with the application follows.

SEQUENCE LISTING (8 sequences)

SEQ ID NO: 1 - DNA, 113 bp, Capsicum baccatum
  source 1..113: /organism="Capsicum baccatum" /mol_type="unassigned DNA"
ttaaactatccttttccaatcaccacatgmccaggcttcgacttgctaaaagctcttttcagcatttgaccctccgcagagagagcggttgaaagcttgtaaacatgaacaag

SEQ ID NO: 2 - DNA, 113 bp, Capsicum annuum
  source 1..113: /organism="Capsicum annuum" /mol_type="unassigned DNA"
ttaaactatccttttccaatcaccacatgmacaggcttcgacttgctaaaagctcttttcagcatttgaccctccgcagagagagcggttgaaagcttgtaaacatgaacaag

SEQ ID NO: 3 - DNA, 100 bp, Capsicum baccatum
  source 1..100: /organism="Capsicum baccatum" /mol_type="unassigned DNA"
gacttgttttgtctgggattgaatgttttttattgttgtagtagtagcagaagcaaaaaatgttgatgtaaattatgaaatattactgctaatatttgtg

SEQ ID NO: 4 - DNA, 100 bp, Capsicum annuum
  source 1..100: /organism="Capsicum annuum" /mol_type="unassigned DNA"
gacttgttttgtctgggattgaatgttttttattgttgtagtagtagcagaagcgaaaaatgttgatgtaaattatgaaatattactgctaatatttgtg

SEQ ID NO: 5 - DNA, 157 bp, Capsicum baccatum
  source 1..157: /organism="Capsicum baccatum" /mol_type="unassigned DNA"
tcagccagtactagttctgctctccaaacctggttaggaaaaaaaacagctacatgaatagtatataatgcactaaaaamytcagatagctaaacgagaacgaacaatagtcactactgggaywsrsaammvdtdttwacactaaatggaaaataca

SEQ ID NO: 6 - DNA, 157 bp, Capsicum annuum
  source 1..157: /organism="Capsicum annuum" /mol_type="unassigned DNA"
tcagccagtactagttctgctctccaaacctggttaggaaaaaaaacagctacatgaatagtatataatgcactaaaaamytcagatagctaaatgagaacgaacaatagtcactactgggaywsrsaammvdtdttwacactaaatggaaaataca

SEQ ID NO: 7 - DNA, 111 bp, Capsicum baccatum
  source 1..111: /organism="Capsicum baccatum" /mol_type="unassigned DNA"
ctgcaccagctctgcttgcactaaaacagaaacgactgacgtttacctggcttgatggggaagcacagaaagtgagcacctctcttcaaatgtttgcattcctttggttaa

SEQ ID NO: 8 - DNA, 111 bp, Capsicum annuum
  source 1..111: /organism="Capsicum annuum" /mol_type="unassigned DNA"
ctgcaccagctctgcttgcactaaaacagaaacgactgacgtttacctggcttgatggggaagcacagaaagtgagcacttctcttcaaatgtttgcattcctttggttaa